European Patent Specification EP 3 517 135 B1, published November 19, 2025. Title: PROMOTERS, EXPRESSION CASSETTES, VECTORS, KITS, AND METHODS FOR THE TREATMENT OF ACHROMATOPSIA AND OTHER DISEASES. Applicant: APPLIED GENETIC TECHNOLOGIES CORPORATION. The sequence listing filed with the application follows.

SEQUENCE LISTING (8 sequences)

SEQ ID NO: 1 - DNA, 1140 bp, Artificial Sequence
  Description of Artificial Sequence: Synthetic polynucleotide
gtgggaccacaaatgagttttcacctggcctggggacacacgtgcccccacaggtgctgagtgactttctaggacagtaatctgctttaggctaaaatgggacttgatcttctgttagccctaatcatcaattagcagagccggtgaaggtgcagaacctaccgcctttccaggcctcctcccacctctgccacctccactctccttcctgggatgtgggggctggcacacgtgtggcccagggcattggtgggattgcactgagctgggtcattagcgtaatcctggacaagggcagacagggcgagcggagggccagctccggggctcaggcaaggctgggggcttcccccagacaccccactcctcctctgctggacccccacttcatagggcacttcgtgttctcaaagggcttccaaatagcatggtggccttggatgcccagggaagcctcagagttgcttatctccctctagacagaaggggaatctcggtcaagagggagaggtcgccctgttcaaggccacccagccagctcatggcggtaatgggacaaggctggccagccatcccaccctcagaagggacccggtggggcaggtgatctcagaggaggctcacttctgggtctcacattcttggatccggttccaggcctcggccctaaatagtctccctgggctttcaagagaaccacatgagaaaggaggattcgggctctgagcagtttcaccacccaccccccagtctgcaaatcctgacccgtgggtccacctgccccaaaggcggacgcaggacagtagaagggaacagagaacacataaacacagagagggccacagcggctcccacagtcaccgccaccttcctggcggggatgggtggggcgtctgagtttggttcccagcaaatccctctgagccgcccttgcgggctcgcctcaggagcaggggagcaagaggtgggaggaggaggtctaagtcccaggcccaattaagagatcaggtagtgtagggtttgggagcttttaaggtgaagaggcccgggctgatcccacaggccagtataaagcgccgtgaccctcaggtgatgcgccagggccggctgccgtcggggacagggctttccatagccatg

SEQ ID NO: 2 - DNA, 1513 bp, Artificial Sequence
  Description of Artificial Sequence: Synthetic polynucleotide
agccatcggctgttagtgacaaagcccctgagtcaagatgacagcagcccccataactcctaatcggctctcccgcgtggagtcatttaggagtagtcgcattagagacaagtccaacatctaatcttccaccctggccagggccccagctggcagcgagggtgggagactccgggcagagcagagggcgctgacattggggcccggcctggcttgggtccctctggcctttccccaggggccctctttccttggggctttcttgggccgccactgctcccgctcctctccccccatcccaccccctcaccccctcgttcttcatatccttctctagtgctccctccactttcatccacccttctgcaagagtgtgggaccacaaatgagttttcacctggcctggggacacacgtgcccccacaggtgctgagtgactttctaggacagtaatctgctttaggctaaaatgggacttgatcttctgttagccctaatcatcaattagcagagccggtgaaggtgcagaacctaccgcctttccaggcctcctcccacctctgccacctccactctccttcctgggatgtgggggctggcacacgtgtggcccagggcattggtgggattgcactgagctgggtcattagcgtaatcctggacaagggcagacagggcgagcggagggccagctccggggctcaggcaaggctgggggcttcccccagacaccccactcctcctctgctggacccccacttcatagggcacttcgtgttctcaaagggcttccaaatagcatggtggccttggatgcccagggaagcctcagagttgcttatctccctctagacagaaggggaatctcggtcaagagggagaggtcgccctgttcaaggccacccagccagctcatggcggtaatgggacaaggctggccagccatcccaccctcagaagggacccggtggggcaggtgatctcagaggaggctcacttctgggtctcacattcttggatccggttccaggcctcggccctaaatagtctccctgggctttcaagagaaccacatgagaaaggaggattcgggctctgagcagtttcaccacccaccccccagtctgcaaatcctgacccgtgggtccacctgccccaaaggcggacgcaggacagtagaagggaacagagaacacataaacacagagagggccacagcggctcccacagtcaccgccaccttcctggcggggatgggtggggcgtctgagtttggttcccagcaaatccctctgagccgcccttgcgggctcgcctcaggagcaggggagcaagaggtgggaggaggaggtctaagtcccaggcccaattaagagatcaggtagtgtagggtttgggagcttttaaggtgaagaggcccgggctgatcccacaggccagtataaagcgccgtgaccctcaggtgatgcgccagggccggctgccgtcggggacagggctttccatagccatg

SEQ ID NO: 3 - DNA, 1727 bp, Artificial Sequence
  Description of Artificial Sequence: Synthetic polynucleotide
ggaggctgaggggtggggaaagggcatgggtgtttcatgaggacagagcttccgtttcatgcaatgaaaagagtttggagacggatggtggtgactggactatacacttacacacggtagcgatggtacactttgtattatgtatattttaccacgatctttttaaagtgtcaaaggcaaatggccaaatggttccttgtcctatagctgtagcagccatcggctgttagtgacaaagcccctgagtcaagatgacagcagcccccataactcctaatcggctctcccgcgtggagtcatttaggagtagtcgcattagagacaagtccaacatctaatcttccaccctggccagggccccagctggcagcgagggtgggagactccgggcagagcagagggcgctgacattggggcccggcctggcttgggtccctctggcctttccccaggggccctctttccttggggctttcttgggccgccactgctcccgctcctctccccccatcccaccccctcaccccctcgttcttcatatccttctctagtgctccctccactttcatccacccttctgcaagagtgtgggaccacaaatgagttttcacctggcctggggacacacgtgcccccacaggtgctgagtgactttctaggacagtaatctgctttaggctaaaatgggacttgatcttctgttagccctaatcatcaattagcagagccggtgaaggtgcagaacctaccgcctttccaggcctcctcccacctctgccacctccactctccttcctgggatgtgggggctggcacacgtgtggcccagggcattggtgggattgcactgagctgggtcattagcgtaatcctggacaagggcagacagggcgagcggagggccagctccggggctcaggcaaggctgggggcttcccccagacaccccactcctcctctgctggacccccacttcatagggcacttcgtgttctcaaagggcttccaaatagcatggtggccttggatgcccagggaagcctcagagttgcttatctccctctagacagaaggggaatctcggtcaagagggagaggtcgccctgttcaaggccacccagccagctcatggcggtaatgggacaaggctggccagccatcccaccctcagaagggacccggtggggcaggtgatctcagaggaggctcacttctgggtctcacattcttggatccggttccaggcctcggccctaaatagtctccctgggctttcaagagaaccacatgagaaaggaggattcgggctctgagcagtttcaccacccaccccccagtctgcaaatcctgacccgtgggtccacctgccccaaaggcggacgcaggacagtagaagggaacagagaacacataaacacagagagggccacagcggctcccacagtcaccgccaccttcctggcggggatgggtggggcgtctgagtttggttcccagcaaatccctctgagccgcccttgcgggctcgcctcaggagcaggggagcaagaggtgggaggaggaggtctaagtcccaggcccaattaagagatcaggtagtgtagggtttgggagcttttaaggtgaagaggcccgggctgatcccacaggccagtataaagcgccgtgaccctcaggtgatgcgccagggccggctgccgtcggggacagggctttccatagccatg

SEQ ID NO: 4 - DNA, 2064 bp, Artificial Sequence
  Description of Artificial Sequence: Synthetic polynucleotide
cccctacagcagccagggtgagattatgaggctgagctgagaatatcaagactgtaccgagtagggggccttggcaagtgtggagagcccggcagctggggcagagggcggagtacggtgtgcgtttacggacctcttcaaacgaggtaggaaggtcagaagtcaaaaagggaacaaatgatgtttaaccacacaaaaatgaaaatccaatggttggatatccattccaaatacacaaaggcaacggataagtgatccgggccaggcacagaaggccatgcacccgtaggattgcactcagagctcccaaatgcataggaatagaagggtgggtgcaggaggctgaggggtggggaaagggcatgggtgtttcatgaggacagagcttccgtttcatgcaatgaaaagagtttggagacggatggtggtgactggactatacacttacacacggtagcgatggtacactttgtattatgtatattttaccacgatctttttaaagtgtcaaaggcaaatggccaaatggttccttgtcctatagctgtagcagccatcggctgttagtgacaaagcccctgagtcaagatgacagcagcccccataactcctaatcggctctcccgcgtggagtcatttaggagtagtcgcattagagacaagtccaacatctaatcttccaccctggccagggccccagctggcagcgagggtgggagactccgggcagagcagagggcgctgacattggggcccggcctggcttgggtccctctggcctttccccaggggccctctttccttggggctttcttgggccgccactgctcccgctcctctccccccatcccaccccctcaccccctcgttcttcatatccttctctagtgctccctccactttcatccacccttctgcaagagtgtgggaccacaaatgagttttcacctggcctggggacacacgtgcccccacaggtgctgagtgactttctaggacagtaatctgctttaggctaaaatgggacttgatcttctgttagccctaatcatcaattagcagagccggtgaaggtgcagaacctaccgcctttccaggcctcctcccacctctgccacctccactctccttcctgggatgtgggggctggcacacgtgtggcccagggcattggtgggattgcactgagctgggtcattagcgtaatcctggacaagggcagacagggcgagcggagggccagctccggggctcaggcaaggctgggggcttcccccagacaccccactcctcctctgctggacccccacttcatagggcacttcgtgttctcaaagggcttccaaatagcatggtggccttggatgcccagggaagcctcagagttgcttatctccctctagacagaaggggaatctcggtcaagagggagaggtcgccctgttcaaggccacccagccagctcatggcggtaatgggacaaggctggccagccatcccaccctcagaagggacccggtggggcaggtgatctcagaggaggctcacttctgggtctcacattcttggatccggttccaggcctcggccctaaatagtctccctgggctttcaagagaaccacatgagaaaggaggattcgggctctgagcagtttcaccacccaccccccagtctgcaaatcctgacccgtgggtccacctgccccaaaggcggacgcaggacagtagaagggaacagagaacacataaacacagagagggccacagcggctcccacagtcaccgccaccttcctggcggggatgggtggggcgtctgagtttggttcccagcaaatccctctgagccgcccttgcgggctcgcctcaggagcaggggagcaagaggtgggaggaggaggtctaagtcccaggcccaattaagagatcaggtagtgtagggtttgggagcttttaaggtgaagaggcccgggctgatcccacaggccagtataaagcgccgtgaccctcaggtgatgcgccagggccggctgccgtcggggacagggctttccatagccatg

SEQ ID NO: 5 - DNA, 44 bp, Artificial Sequence
  Description of Artificial Sequence: Synthetic primer
gatttaagcttgcggccgcgggtacaattccgcagcttttagag

SEQ ID NO: 6 - DNA, 27 bp, Artificial Sequence
  Description of Artificial Sequence: Synthetic primer
ctgcaagcttgtgggaccacaaatcag

SEQ ID NO: 7 - DNA, 26 bp, Artificial Sequence
  Description of Artificial Sequence: Synthetic primer
tagcggtaccagccatcggctgttag

SEQ ID NO: 8 - DNA, 24 bp, Artificial Sequence
  Description of Artificial Sequence: Synthetic primer
gtgggtaccggaggctgaggggtg